European Patent Application EP 4 506 362 A1, published February 12, 2025. Title: CD80 PROTEIN VARIANT AND CD80 FUSION PROTEIN. Applicant: HANGZHOU SUMGEN BIOTECH CO., LTD. The sequence listing filed with the application follows.

SEQUENCE LISTING (37 sequences)

SEQ ID NO: 1 - protein, 209 aa, synthetic construct
  REGION 1..209: note = wild type CD80 ECD
VIHVTKEVKEVATLSCGHNVSVEELAQTRIYWQKEKKMVLTMMSGDMNIWPEYKNRTIFDITNNLSIVILALRPSDEGTYECVVLKYEKDAFKREHLAEVTLSVKADFPTPSISDFEIPTSNIRRIICSTSGGFPEPHLSWLENGEELNAINTTVSQDPETELYAVSSKLDFNMTTNHSFMCLIKYGHLRVNQTFNWNTTKQEHFPDNL

SEQ ID NO: 2 - protein, 106 aa, synthetic construct
  REGION 1..106: note = wild type CD80 IgV
VIHVTKEVKEVATLSCGHNVSVEELAQTRIYWQKEKKMVLTMMSGDMNIWPEYKNRTIFDITNNLSIVILALRPSDEGTYECVVLKYEKDAFKREHLAEVTLSVKA

SEQ ID NO: 3 - protein, 106 aa, synthetic construct
  REGION 1..106: note = M09
VIHVTKEVKEVATLSCGHAVSVEELAQTRIYWQKEKKMVLTMMSGDMNIWPEYKNRTIFDITNNLSIVILALRPSDEGTYECVVLKYEKDAFKREHLAEVTLSVKA

SEQ ID NO: 4 - protein, 106 aa, synthetic construct
  REGION 1..106: note = M10
VIHVTKEVKEVATLSCGHNVSVEELAQTRIYWQKEKKMVLTMMSGDMNIWPEYKARTIFDITNNLSIVILALRPSDEGTYECVVLKYEKDAFKREHLAEVTLSVKA

SEQ ID NO: 5 - protein, 106 aa, synthetic construct
  REGION 1..106: note = M11
VIHVTKEVKEVATLSCGHNVSVEELAQTRIYWQKEKKMVLTMMSGDMNIWPEYKNRTIFDITNALSIVILALRPSDEGTYECVVLKYEKDAFKREHLAEVTLSVKA

SEQ ID NO: 6 - protein, 209 aa, synthetic construct
  REGION 1..209: note = M12
VIHVTKEVKEVATLSCGHNVSVEELAQTRIYWQKEKKMVLTMMSGDMNIWPEYKARTIFDITNALSIVILALRPSDEGTYECVVLKYEKDAFKREHLAEVTLSVKADFPTPSISDFEIPTSNIRRIICSTSGGFPEPHLSWLENGEELNAINTTVSQDPETELYAVSSKLDFNMTTNHSFMCLIKYGHLRVNQTFNWNTTKQEHFPDNL

SEQ ID NO: 7 - protein, 209 aa, synthetic construct
  REGION 1..209: note = M13
VIHVTKEVKEVATLSCGHNVSVEELAQTRIYWQKEKKMVLTMMSGDMNIWPEYKARTIFDITNALSIVILALRPSDEGTYECVVLKYEKDAFKREHLAEVTLSVKADFPTPSISDFEIPTSNIRRIICSTSGGFPEPHLSWLENGEELNAIATTVSQDPETELYAVSSKLDFNMTTNHSFMCLIKYGHLRVAQTFNWATTKQEHFPDNL

SEQ ID NO: 8 - protein, 209 aa, synthetic construct
  REGION 1..209: note = M14
VIHVTKEVKEVATLSCGHNVSVEELAQTRIYWQKEKKMVLTMMSGDMNIWPEYKARTIFDITNALSIVILALRPSDEGTYECVVLKYEKDAFKREHLAEVTLSVKADFPTPSISDFEIPTSNIRRIICSTSGGFPEPHLSWLENGEELNAIATTVSQDPETELYAVSSKLDFNMTTNHSFMCLIKYGHLRVNQTFNWNTTKQEHFPDNL

SEQ ID NO: 9 - protein, 209 aa, synthetic construct
  REGION 1..209: note = M15
VIHVTKEVKEVATLSCGHNVSVEELAQTRIYWQKEKKMVLTMMSGDMNIWPEYKARTIFDITNALSIVILALRPSDEGTYECVVLKYEKDAFKREHLAEVTLSVKADFPTPSISDFEIPTSNIRRIICSTSGGFPEPHLSWLENGEELNAINTTVSQDPETELYAVSSKLDFNMTTNHSFMCLIKYGHLRVAQTFNWNTTKQEHFPDNL

SEQ ID NO: 10 - protein, 209 aa, synthetic construct
  REGION 1..209: note = M16
VIHVTKEVKEVATLSCGHNVSVEELAQTRIYWQKEKKMVLTMMSGDMNIWPEYKARTIFDITNALSIVILALRPSDEGTYECVVLKYEKDAFKREHLAEVTLSVKADFPTPSISDFEIPTSNIRRIICSTSGGFPEPHLSWLENGEELNAINTTVSQDPETELYAVSSKLDFNMTTNHSFMCLIKYGHLRVNQTFNWATTKQEHFPDNL

SEQ ID NO: 11 - protein, 209 aa, synthetic construct
  REGION 1..209: note = M18
VIHVTKEVKEVATLSCGHAVSVEELAQTRIYWQKEKKMVLTMMSGDMNIWPEYKARTIFDITNALSIVILALRPSDEGTYECVVLKYEKDAFKREHLAEVTLSVKADFPTPSISDFEIPTSNIRRIICSTSGGFPEPHLSWLENGEELNAINTTVSQDPETELYAVSSKLDFNMTTNHSFMCLIKYGHLRVNQTFNWNTTKQEHFPDNL

SEQ ID NO: 12 - protein, 209 aa, synthetic construct
  REGION 1..209: note = M19
VIHVTKEVKEVATLSCGHAVSVEELAQTRIYWQKEKKMVLTMMSGDMNIWPEYKARTIFDITNALSIVILALRPSDEGTYECVVLKYEKDAFKREHLAEVTLSVKADFPTPSISDFEIPTSNIRRIICSTSGGFPEPHLSWLENGEELNAIATTVSQDPETELYAVSSKLDFNMTTNHSFMCLIKYGHLRVAQTFNWATTKQEHFPDNL

SEQ ID NO: 13 - protein, 209 aa, synthetic construct
  REGION 1..209: note = M20
VIHVTKEVKEVATLSCGHAVSVEELAQTRIYWQKEKKMVLTMMSGDMNIWPEYKNRTIFDITNALSIVILALRPSDEGTYECVVLKYEKDAFKREHLAEVTLSVKADFPTPSISDFEIPTSNIRRIICSTSGGFPEPHLSWLENGEELNAIATTVSQDPETELYAVSSKLDFNMTTNHSFMCLIKYGHLRVAQTFNWATTKQEHFPDNL

SEQ ID NO: 14 - protein, 209 aa, synthetic construct
  REGION 1..209: note = M21
VIHVTKEVKEVATLSCGHAVSVEELAQTRIYWQKEKKMVLTMMSGDMNIWPEYKARTIFDITNNLSIVILALRPSDEGTYECVVLKYEKDAFKREHLAEVTLSVKADFPTPSISDFEIPTSNIRRIICSTSGGFPEPHLSWLENGEELNAIATTVSQDPETELYAVSSKLDFNMTTNHSFMCLIKYGHLRVAQTFNWATTKQEHFPDNL

SEQ ID NO: 15 - protein, 209 aa, synthetic construct
  REGION 1..209: note = M22
VIHVTKEVKEVATLSCGHAVSVEELAQTRIYWQKEKKMVLTMMSGDMNIWPEYKARTIFDITNALSIVILALRPSDEGTYECVVLKYEKDAFKREHLAEVTLSVKADFPTPSISDFEIPTSNIRRIICSTSGGFPEPHLSWLENGEELNAINTTVSQDPETELYAVSSKLDFNMTTNHSFMCLIKYGHLRVAQTFNWATTKQEHFPDNL

SEQ ID NO: 16 - protein, 209 aa, synthetic construct
  REGION 1..209: note = M23
VIHVTKEVKEVATLSCGHAVSVEELAQTRIYWQKEKKMVLTMMSGDMNIWPEYKARTIFDITNALSIVILALRPSDEGTYECVVLKYEKDAFKREHLAEVTLSVKADFPTPSISDFEIPTSNIRRIICSTSGGFPEPHLSWLENGEELNAIATTVSQDPETELYAVSSKLDFNMTTNHSFMCLIKYGHLRVNQTFNWATTKQEHFPDNL

SEQ ID NO: 17 - protein, 209 aa, synthetic construct
  REGION 1..209: note = M24
VIHVTKEVKEVATLSCGHAVSVEELAQTRIYWQKEKKMVLTMMSGDMNIWPEYKARTIFDITNALSIVILALRPSDEGTYECVVLKYEKDAFKREHLAEVTLSVKADFPTPSISDFEIPTSNIRRIICSTSGGFPEPHLSWLENGEELNAIATTVSQDPETELYAVSSKLDFNMTTNHSFMCLIKYGHLRVAQTFNWNTTKQEHFPDNL

SEQ ID NO: 18 - protein, 209 aa, synthetic construct
  REGION 1..209: note = M25
VIHVTKEVKEVATLSCGHNVSVEELAQTRIYWQKEKKMVLTMMSGDMNIWPEYKARTIFDITNALSIVILALRPSDEGTYECVVLKYEKDAFKREHLAEVTLSVKADFPTPSISDFEIPTSNIRRIICSTSGGFPEPHLSWLENGEELNAINTTVSQDPETELYAVSSKLDFNMTTNHSFMCLIKYGHLRVAQTFNWATTKQEHFPDNL

SEQ ID NO: 19 - protein, 209 aa, synthetic construct
  REGION 1..209: note = M26
VIHVTKEVKEVATLSCGHNVSVEELAQTRIYWQKEKKMVLTMMSGDMNIWPEYKARTIFDITNALSIVILALRPSDEGTYECVVLKYEKDAFKREHLAEVTLSVKADFPTPSISDFEIPTSNIRRIICSTSGGFPEPHLSWLENGEELNAIATTVSQDPETELYAVSSKLDFNMTTNHSFMCLIKYGHLRVNQTFNWATTKQEHFPDNL

SEQ ID NO: 20 - protein, 209 aa, synthetic construct
  REGION 1..209: note = M27
VIHVTKEVKEVATLSCGHNVSVEELAQTRIYWQKEKKMVLTMMSGDMNIWPEYKARTIFDITNALSIVILALRPSDEGTYECVVLKYEKDAFKREHLAEVTLSVKADFPTPSISDFEIPTSNIRRIICSTSGGFPEPHLSWLENGEELNAIATTVSQDPETELYAVSSKLDFNMTTNHSFMCLIKYGHLRVAQTFNWNTTKQEHFPDNL

SEQ ID NO: 21 - protein, 209 aa, synthetic construct
  REGION 1..209: note = M28
VIHVTKEVKEVATLSCGHNVSVEELAQTRIYWQKEKKMVLTMMSGDMNIWPEYKQRTIFDITNALSIVILALRPSDEGTYECVVLKYEKDAFKREHLAEVTLSVKADFPTPSISDFEIPTSNIRRIICSTSGGFPEPHLSWLENGEELNAIATTVSQDPETELYAVSSKLDFNMTTNHSFMCLIKYGHLRVNQTFNWQTTKQEHFPDNL

SEQ ID NO: 22 - protein, 209 aa, synthetic construct
  REGION 1..209: note = M29
VIHVTKEVKEVATLSCGHNVSVEELAQTRIYWQKEKKMVLTMMSGDMNIWPEYKQRTIFDITNALSIVILALRPSDEGTYECVVLKYEKDAFKREHLAEVTLSVKADFPTPSISDFEIPTSNIRRIICSTSGGFPEPHLSWLENGEELNAIATTVSQDPETELYAVSSKLDFQMTTAHSFMCLIKYGHLRVNQTFNWQTTKQEHFPDNL

SEQ ID NO: 23 - protein, 209 aa, synthetic construct
  REGION 1..209: note = M30
VIHVTKEVKEVATLSCGHNVSVEELAQTRIYWQKEKKMVLTMMSGDMNIWPEYKQRTIFDITNALSIVILALRPSDEGTYECVVLKYEKDAFKREHLAEVTLSVKADFPTPSISDFEIPTSNIRRIICSTSGGFPEPHLSWLENGEELNAIATTVSQDPETELYAVSSKLDFQMTTNHSFMCLIKYGHLRVNQTFNWQTTKQEHFPDNL

SEQ ID NO: 24 - protein, 209 aa, synthetic construct
  REGION 1..209: note = M31
VIHVTKEVKEVATLSCGHNVSVEELAQTRIYWQKEKKMVLTMMSGDMNIWPEYKQRTIFDITNALSIVILALRPSDEGTYECVVLKYEKDAFKREHLAEVTLSVKADFPTPSISDFEIPTSNIRRIICSTSGGFPEPHLSWLENGEELNAIATTVSQDPETELYAVSSKLDFNMTTAHSFMCLIKYGHLRVNQTFNWQTTKQEHFPDNL

SEQ ID NO: 25 - protein, 232 aa, synthetic construct
  REGION 1..232: note = human IgG1 Fc
EPKSCDKTHTCPPCPAPELLGGPSVFLFPPKPKDTLMISRTPEVTCVVVDVSHEDPEVKFNWYVDGVEVHNAKTKPREEQYNSTYRVVSVLTVLHQDWLNGKEYKCKVSNKALPAPIEKTISKAKGQPREPQVYTLPPSRDELTKNQVSLTCLVKGFYPSDIAVEWESNGQPENNYKTTPPVLDSDGSFFLYSKLTVDKSRWQQGNVFSCSVMHEALHNHYTQKSLSLSPGK

SEQ ID NO: 26 - protein, 229 aa, synthetic construct
  REGION 1..229: note = human IgG4 Fc
ESKYGPPCPPCPAPEFLGGPSVFLFPPKPKDTLMISRTPEVTCVVVDVSQEDPEVQFNWYVDGVEVHNAKTKPREEQFNSTYRVVSVLTVLHQDWLNGKEYKCKVSNKGLPSSIEKTISKAKGQPREPQVYTLPPSQEEMTKNQVSLTCLVKGFYPSDIAVEWESNGQPENNYKTTPPVLDSDGSFFLYSRLTVDKSRWQEGNVFSCSVMHEALHNHYTQKSLSLSLGK

SEQ ID NO: 27 - protein, 338 aa, synthetic construct
  REGION 1..338: note = CD80M11
VIHVTKEVKEVATLSCGHNVSVEELAQTRIYWQKEKKMVLTMMSGDMNIWPEYKNRTIFDITNALSIVILALRPSDEGTYECVVLKYEKDAFKREHLAEVTLSVKAEPKSCDKTHTCPPCPAPELLGGPSVFLFPPKPKDTLMISRTPEVTCVVVDVSHEDPEVKFNWYVDGVEVHNAKTKPREEQYNSTYRVVSVLTVLHQDWLNGKEYKCKVSNKALPAPIEKTISKAKGQPREPQVYTLPPSRDELTKNQVSLTCLVKGFYPSDIAVEWESNGQPENNYKTTPPVLDSDGSFFLYSKLTVDKSRWQQGNVFSCSVMHEALHNHYTQKSLSLSPGK

SEQ ID NO: 28 - protein, 441 aa, synthetic construct
  REGION 1..441: note = CD80M12
VIHVTKEVKEVATLSCGHNVSVEELAQTRIYWQKEKKMVLTMMSGDMNIWPEYKARTIFDITNALSIVILALRPSDEGTYECVVLKYEKDAFKREHLAEVTLSVKADFPTPSISDFEIPTSNIRRIICSTSGGFPEPHLSWLENGEELNAINTTVSQDPETELYAVSSKLDFNMTTNHSFMCLIKYGHLRVNQTFNWNTTKQEHFPDNLEPKSCDKTHTCPPCPAPELLGGPSVFLFPPKPKDTLMISRTPEVTCVVVDVSHEDPEVKFNWYVDGVEVHNAKTKPREEQYNSTYRVVSVLTVLHQDWLNGKEYKCKVSNKALPAPIEKTISKAKGQPREPQVYTLPPSRDELTKNQVSLTCLVKGFYPSDIAVEWESNGQPENNYKTTPPVLDSDGSFFLYSKLTVDKSRWQQGNVFSCSVMHEALHNHYTQKSLSLSPGK

SEQ ID NO: 29 - protein, 441 aa, synthetic construct
  REGION 1..441: note = CD80M14
VIHVTKEVKEVATLSCGHNVSVEELAQTRIYWQKEKKMVLTMMSGDMNIWPEYKARTIFDITNALSIVILALRPSDEGTYECVVLKYEKDAFKREHLAEVTLSVKADFPTPSISDFEIPTSNIRRIICSTSGGFPEPHLSWLENGEELNAIATTVSQDPETELYAVSSKLDFNMTTNHSFMCLIKYGHLRVNQTFNWNTTKQEHFPDNLEPKSCDKTHTCPPCPAPELLGGPSVFLFPPKPKDTLMISRTPEVTCVVVDVSHEDPEVKFNWYVDGVEVHNAKTKPREEQYNSTYRVVSVLTVLHQDWLNGKEYKCKVSNKALPAPIEKTISKAKGQPREPQVYTLPPSRDELTKNQVSLTCLVKGFYPSDIAVEWESNGQPENNYKTTPPVLDSDGSFFLYSKLTVDKSRWQQGNVFSCSVMHEALHNHYTQKSLSLSPGK

SEQ ID NO: 30 - protein, 441 aa, synthetic construct
  REGION 1..441: note = CD80M15
VIHVTKEVKEVATLSCGHNVSVEELAQTRIYWQKEKKMVLTMMSGDMNIWPEYKARTIFDITNALSIVILALRPSDEGTYECVVLKYEKDAFKREHLAEVTLSVKADFPTPSISDFEIPTSNIRRIICSTSGGFPEPHLSWLENGEELNAINTTVSQDPETELYAVSSKLDFNMTTNHSFMCLIKYGHLRVAQTFNWNTTKQEHFPDNLEPKSCDKTHTCPPCPAPELLGGPSVFLFPPKPKDTLMISRTPEVTCVVVDVSHEDPEVKFNWYVDGVEVHNAKTKPREEQYNSTYRVVSVLTVLHQDWLNGKEYKCKVSNKALPAPIEKTISKAKGQPREPQVYTLPPSRDELTKNQVSLTCLVKGFYPSDIAVEWESNGQPENNYKTTPPVLDSDGSFFLYSKLTVDKSRWQQGNVFSCSVMHEALHNHYTQKSLSLSPGK

SEQ ID NO: 31 - protein, 441 aa, synthetic construct
  REGION 1..441: note = CD80M16
VIHVTKEVKEVATLSCGHNVSVEELAQTRIYWQKEKKMVLTMMSGDMNIWPEYKARTIFDITNALSIVILALRPSDEGTYECVVLKYEKDAFKREHLAEVTLSVKADFPTPSISDFEIPTSNIRRIICSTSGGFPEPHLSWLENGEELNAINTTVSQDPETELYAVSSKLDFNMTTNHSFMCLIKYGHLRVNQTFNWATTKQEHFPDNLEPKSCDKTHTCPPCPAPELLGGPSVFLFPPKPKDTLMISRTPEVTCVVVDVSHEDPEVKFNWYVDGVEVHNAKTKPREEQYNSTYRVVSVLTVLHQDWLNGKEYKCKVSNKALPAPIEKTISKAKGQPREPQVYTLPPSRDELTKNQVSLTCLVKGFYPSDIAVEWESNGQPENNYKTTPPVLDSDGSFFLYSKLTVDKSRWQQGNVFSCSVMHEALHNHYTQKSLSLSPGK

SEQ ID NO: 32 - protein, 441 aa, synthetic construct
  REGION 1..441: note = CD80M26
VIHVTKEVKEVATLSCGHNVSVEELAQTRIYWQKEKKMVLTMMSGDMNIWPEYKARTIFDITNALSIVILALRPSDEGTYECVVLKYEKDAFKREHLAEVTLSVKADFPTPSISDFEIPTSNIRRIICSTSGGFPEPHLSWLENGEELNAIATTVSQDPETELYAVSSKLDFNMTTNHSFMCLIKYGHLRVNQTFNWATTKQEHFPDNLEPKSCDKTHTCPPCPAPELLGGPSVFLFPPKPKDTLMISRTPEVTCVVVDVSHEDPEVKFNWYVDGVEVHNAKTKPREEQYNSTYRVVSVLTVLHQDWLNGKEYKCKVSNKALPAPIEKTISKAKGQPREPQVYTLPPSRDELTKNQVSLTCLVKGFYPSDIAVEWESNGQPENNYKTTPPVLDSDGSFFLYSKLTVDKSRWQQGNVFSCSVMHEALHNHYTQKSLSLSPGK

SEQ ID NO: 33 - protein, 441 aa, synthetic construct
  REGION 1..441: note = CD80M27
VIHVTKEVKEVATLSCGHNVSVEELAQTRIYWQKEKKMVLTMMSGDMNIWPEYKARTIFDITNALSIVILALRPSDEGTYECVVLKYEKDAFKREHLAEVTLSVKADFPTPSISDFEIPTSNIRRIICSTSGGFPEPHLSWLENGEELNAIATTVSQDPETELYAVSSKLDFNMTTNHSFMCLIKYGHLRVAQTFNWNTTKQEHFPDNLEPKSCDKTHTCPPCPAPELLGGPSVFLFPPKPKDTLMISRTPEVTCVVVDVSHEDPEVKFNWYVDGVEVHNAKTKPREEQYNSTYRVVSVLTVLHQDWLNGKEYKCKVSNKALPAPIEKTISKAKGQPREPQVYTLPPSRDELTKNQVSLTCLVKGFYPSDIAVEWESNGQPENNYKTTPPVLDSDGSFFLYSKLTVDKSRWQQGNVFSCSVMHEALHNHYTQKSLSLSPGK

SEQ ID NO: 34 - protein, 441 aa, synthetic construct
  REGION 1..441: note = CD80M28
VIHVTKEVKEVATLSCGHNVSVEELAQTRIYWQKEKKMVLTMMSGDMNIWPEYKQRTIFDITNALSIVILALRPSDEGTYECVVLKYEKDAFKREHLAEVTLSVKADFPTPSISDFEIPTSNIRRIICSTSGGFPEPHLSWLENGEELNAIATTVSQDPETELYAVSSKLDFNMTTNHSFMCLIKYGHLRVNQTFNWQTTKQEHFPDNLEPKSCDKTHTCPPCPAPELLGGPSVFLFPPKPKDTLMISRTPEVTCVVVDVSHEDPEVKFNWYVDGVEVHNAKTKPREEQYNSTYRVVSVLTVLHQDWLNGKEYKCKVSNKALPAPIEKTISKAKGQPREPQVYTLPPSRDELTKNQVSLTCLVKGFYPSDIAVEWESNGQPENNYKTTPPVLDSDGSFFLYSKLTVDKSRWQQGNVFSCSVMHEALHNHYTQKSLSLSPGK

SEQ ID NO: 35 - protein, 441 aa, synthetic construct
  REGION 1..441: note = CD80M29
VIHVTKEVKEVATLSCGHNVSVEELAQTRIYWQKEKKMVLTMMSGDMNIWPEYKQRTIFDITNALSIVILALRPSDEGTYECVVLKYEKDAFKREHLAEVTLSVKADFPTPSISDFEIPTSNIRRIICSTSGGFPEPHLSWLENGEELNAIATTVSQDPETELYAVSSKLDFQMTTAHSFMCLIKYGHLRVNQTFNWQTTKQEHFPDNLEPKSCDKTHTCPPCPAPELLGGPSVFLFPPKPKDTLMISRTPEVTCVVVDVSHEDPEVKFNWYVDGVEVHNAKTKPREEQYNSTYRVVSVLTVLHQDWLNGKEYKCKVSNKALPAPIEKTISKAKGQPREPQVYTLPPSRDELTKNQVSLTCLVKGFYPSDIAVEWESNGQPENNYKTTPPVLDSDGSFFLYSKLTVDKSRWQQGNVFSCSVMHEALHNHYTQKSLSLSPGK

SEQ ID NO: 36 - protein, 441 aa, synthetic construct
  REGION 1..441: note = CD80M30
VIHVTKEVKEVATLSCGHNVSVEELAQTRIYWQKEKKMVLTMMSGDMNIWPEYKQRTIFDITNALSIVILALRPSDEGTYECVVLKYEKDAFKREHLAEVTLSVKADFPTPSISDFEIPTSNIRRIICSTSGGFPEPHLSWLENGEELNAIATTVSQDPETELYAVSSKLDFQMTTNHSFMCLIKYGHLRVNQTFNWQTTKQEHFPDNLEPKSCDKTHTCPPCPAPELLGGPSVFLFPPKPKDTLMISRTPEVTCVVVDVSHEDPEVKFNWYVDGVEVHNAKTKPREEQYNSTYRVVSVLTVLHQDWLNGKEYKCKVSNKALPAPIEKTISKAKGQPREPQVYTLPPSRDELTKNQVSLTCLVKGFYPSDIAVEWESNGQPENNYKTTPPVLDSDGSFFLYSKLTVDKSRWQQGNVFSCSVMHEALHNHYTQKSLSLSPGK

SEQ ID NO: 37 - protein, 441 aa, synthetic construct
  REGION 1..441: note = CD80M31
VIHVTKEVKEVATLSCGHNVSVEELAQTRIYWQKEKKMVLTMMSGDMNIWPEYKQRTIFDITNALSIVILALRPSDEGTYECVVLKYEKDAFKREHLAEVTLSVKADFPTPSISDFEIPTSNIRRIICSTSGGFPEPHLSWLENGEELNAIATTVSQDPETELYAVSSKLDFNMTTAHSFMCLIKYGHLRVNQTFNWQTTKQEHFPDNLEPKSCDKTHTCPPCPAPELLGGPSVFLFPPKPKDTLMISRTPEVTCVVVDVSHEDPEVKFNWYVDGVEVHNAKTKPREEQYNSTYRVVSVLTVLHQDWLNGKEYKCKVSNKALPAPIEKTISKAKGQPREPQVYTLPPSRDELTKNQVSLTCLVKGFYPSDIAVEWESNGQPENNYKTTPPVLDSDGSFFLYSKLTVDKSRWQQGNVFSCSVMHEALHNHYTQKSLSLSPGK